European Patent Specification EP 4 063 502 B1, published June 4, 2025. Title: Novel cysteine sulfinate desulfinase variant and a method for producing L-valine using the same. Applicant: CJ CheilJedang Corporation. The sequence listing filed with the application follows.

SEQUENCE LISTING (11 sequences)

SEQ ID NO: 1 - protein, 358 aa, Artificial Sequence
  Cysteine sulfinate desulfinase variant
MLYLDNAATTSVRKEALEAMWPYLTGAFGNPSSPHEVGRLASAGLEDARARVARIIGGRPTQMTFTSGGSEANNLAIKGACLANPRGRHLITTPIEHDSVLETAAYLERFHDFEITYLSPDHTGLISPEDLRKAVRPDTTLISIGYANNEVGTIQPIAELAAVSSTPFHTDAVQAAHLTFDLGVDALSLSGHKFGAPKGIGVLWSKLPLEPVIHGGGQEKGRRSGTENVAGAVAFATALELARAESYPDLGEFIEEVLTIPGAHLTGHPRMRIDGHASFLFDSIGSETVLLELERQGIVCSSGSACGSGEVSHVLLALGLEEDQARTAVRCTFSTTHSREDALVAASALKSAVALIRG

SEQ ID NO: 2 - DNA, 1077 bp, Artificial Sequence
  Cysteine sulfinate desulfinase variant coding gene
atgctctaccttgataatgcagccaccaccagtgtgcgcaaagaagcacttgaggccatgtggccttatctcaccggagcgtttggcaatccgtcaagccctcatgaggtgggaagactcgcctctgcgggtctagaagatgctcgagctcgggtggcccgcattatcggaggacgccccacacagatgacgtttacgtcgggtggatcagaagccaacaacctcgctatcaaaggagcgtgcttagctaatcctcgtggccggcacctcatcactaccccgatcgagcatgacagtgtcctagaaactgctgcttatcttgaaaggtttcatgatttcgagatcacctacctatcccccgatcacactgggctgatctccccggaggatctccgcaaagcagtcaggccggacaccacattgatcagcattggttatgccaacaatgaggtgggaaccattcagccgatagctgagttagcggcggtaagcagtacgccttttcacaccgatgcagtgcaagctgcacatttaacctttgacttgggagttgacgcgttaagtttgtcgggtcataaattcggtgcgcctaaagggattggagtgttgtggtcaaagcttcccctggagccggtaatccatggcggcggccaggaaaaagggcggcgtagtggcacggaaaacgttgcgggggctgtcgcctttgccactgccttggaattggccagggcggaatcctatccagatcttggcgaattcatcgaggaagttctcactatcccgggagcacacctgactggacatcctaggatgcgcattgatggacacgcatcttttctcttcgacagcataggatctgaaactgttcttctggaattggaacgccaaggcattgtctgctcctctggatctgcctgtggttccggtgaggtatcccatgtgttgctggcgttggggcttgaggaggatcaagcacgaacggctgtgcgctgtacttttagtacaacacacagccgtgaagatgcgctcgtggcagcctctgctcttaaatccgcggtcgccttaatcagagggtga

SEQ ID NO: 3 - protein, 358 aa, Artificial Sequence
  Wild-type cysteine sulfinate desulfinase
MLYLDNAATTSVRKEALEAMWPYLTGAFGNPSSPHEVGRLASAGLEDARARVARIIGGRPTQMTFTSGGSEANNLAIKGACLANPRGRHLITTPIEHDSVLETAAYLERFHDFEITYLSPDHTGLISPEDLRKAVRPDTTLISIGYANNEVGTIQPIAELAAVSSTPFHTDAVQAAHLTFDLGVDALSLSGHKFGAPKGIGVLWSKLPLEPVIHGGGQEKGRRSGTENVAGAVAFATALELARAESYPDLGEFIEEVLTIPGAHLTGHPRMRIDGHASFLFDSIGSETVLLELERQGIVCSPGSACGSGEVSHVLLALGLEEDQARTAVRCTFSTTHSREDALVAASALKSAVALIRG

SEQ ID NO: 4 - DNA, 1077 bp, Artificial Sequence
  Wild-type cysteine sulfinate desulfinase coding gene
atgctctaccttgataatgcagccaccaccagtgtgcgcaaagaagcacttgaggccatgtggccttatctcaccggagcgtttggcaatccgtcaagccctcatgaggtgggaagactcgcctctgcgggtctagaagatgctcgagctcgggtggcccgcattatcggaggacgccccacacagatgacgtttacgtcgggtggatcagaagccaacaacctcgctatcaaaggagcgtgcttagctaatcctcgtggccggcacctcatcactaccccgatcgagcatgacagtgtcctagaaactgctgcttatcttgaaaggtttcatgatttcgagatcacctacctatcccccgatcacactgggctgatctccccggaggatctccgcaaagcagtcaggccggacaccacattgatcagcattggttatgccaacaatgaggtgggaaccattcagccgatagctgagttagcggcggtaagcagtacgccttttcacaccgatgcagtgcaagctgcacatttaacctttgacttgggagttgacgcgttaagtttgtcgggtcataaattcggtgcgcctaaagggattggagtgttgtggtcaaagcttcccctggagccggtaatccatggcggcggccaggaaaaagggcggcgtagtggcacggaaaacgttgcgggggctgtcgcctttgccactgccttggaattggccagggcggaatcctatccagatcttggcgaattcatcgaggaagttctcactatcccgggagcacacctgactggacatcctaggatgcgcattgatggacacgcatcttttctcttcgacagcataggatctgaaactgttcttctggaattggaacgccaaggcattgtctgctcccctggatctgcctgtggttccggtgaggtatcccatgtgttgctggcgttggggcttgaggaggatcaagcacgaacggctgtgcgctgtacttttagtacaacacacagccgtgaagatgcgctcgtggcagcctctgctcttaaatccgcggtcgccttaatcagagggtga

SEQ ID NO: 5 - DNA, 36 bp, Artificial Sequence
  nadS_1F
tcgagctcggtaccccagtcaggccggacaccacat

SEQ ID NO: 6 - DNA, 44 bp, Artificial Sequence
  nadS_2R
ccggaaccacaggcagatccagaggagcagacaatgccttggcg

SEQ ID NO: 7 - DNA, 44 bp, Artificial Sequence
  nadS_3F
cgccaaggcattgtctgctcctctggatctgcctgtggttccgg

SEQ ID NO: 8 - DNA, 36 bp, Artificial Sequence
  nadS_4R
ctctagaggatcccctgatgccagcagtgcagtcca

SEQ ID NO: 9 - DNA, 21 bp, Artificial Sequence
  nadS_5F
cagtcaggccggacaccacat

SEQ ID NO: 10 - DNA, 21 bp, Artificial Sequence
  nadS_6R
tgatgccagcagtgcagtcca

SEQ ID NO: 11 - DNA, 5803 bp, Artificial Sequence
  pDCM2
gttcgcttgctgtccataaaaccgcccagtctagctatcgccatgtaagcccactgcaagctacctgctttctctttgcgcttgcgttttcccttgtccagatagcccagtagctgacattcatccggggtcagcaccgtttctgcggactggctttctacgtgttccgcttcctttagcagcccttgcgccctgagtgcttgcggcagcgtgaagctagcttttatcgccattcgccattcaggctgcgcaactgttgggaagggcgatcggtgcgggcctcttcgctattacgccagctggcgaaagggggatgtgctgcaaggcgattaagttgggtaacgccagggttttcccagtcacgacgttgtaaaacgacggccagtgaattcgagctcggtacccggggatcctctagagtcgacctgcaggcatgcaagcttggcgtaatcatggtcatagctgtttcctgtgtgaaattgttatccgctcacaattccacacaacatacgagccggaagcataaagtgtaaagcctggggtgcctaatgagtgagctaactcacattaattgcgttgcgctcactgcccgctttccagtcgggaaacctgtcgtgccagctgcattaatgaatcggccaacgcgcggggagaggcggtttgcgtattgggcgctcttccgcttcctcgctcactgactcgctgcgctcggtcgttcggctgcggcgagcggtatcagctcactcaaaggcggtaatacggttatccacagaatcaggggataacgcaggaaagaacatgtgagcaaaaggccagcaaaaggccaggaaccgtaaaaaggccgcgttgctggcgtttttccataggctccgcccccctgacgagcatcacaaaaatcgacgctcaagtcagaggtggcgaaacccgacaggactataaagataccaggcgtttccccctggaagctccctcgtgcgctctcctgttccgaccctgccgcttaccggatacctgtccgcctttctcccttcgggaagcgtggcgctttctcaatgctcacgctgtaggtatctcagttcggtgtaggtcgttcgctccaagctgggctgtgtgcacgaaccccccgttcagcccgaccgctgcgccttatccggtaactatcgtcttgagtccaacccggtaagacacgacttatcgccactggcagcagccactggtaacaggattagcagagcgaggtatgtaggcggtgctacagagttcttgaagtggtggcctaactacggctacactagaaggacagtatttggtatctgcgctctgctgaagccagttaccttcggaaaaagagttggtagctcttgatccggcaaacaaaccaccgctggtagcggtggtttttttgtttgcaagcagcagattacgcgcagaaaaaaaggatctcaagaagatcctttgatcttttctacggggtctgacgctcagtggaacgaaaactcacgttaagggattttggtcatgagattatcaaaaaggatcttcacctagatccttttggggtgggcgaagaactccagcatgagatccccgcgctggaggatcatccagccctgatagaaacagaagccactggagcacctcaaaaacaccatcatacactaaatcagtaagttggcagcatcacccgacgcactttgcgccgaataaatacctgtgacggaagatcacttcgcagaataaataaatcctggtgtccctgttgataccgggaagccctgggccaacttttggcgaaaatgagacgttgatcggcacgtaagaggttccaactttcaccataatgaaataagatcactaccgggcgtattttttgagttatcgagattttcaggagctgatagaaacagaagccactggagcacctcaaaaacaccatcatacactaaatcagtaagttggcagcatcacccgacgcactttgcgccgaataaatacctgtgacggaagatcacttcgcagaataaataaatcctggtgtccctgttgataccgggaagccctgggccaacttttggcgaaaatgagacgttgatcggcacgtaagaggttccaactttcaccataatgaaataagatcactaccgggcgtattttttgagttatcgagattttcaggagctctttggcatcgtctctcgcctgtcccctcagttcagtaatttcctgcatttgcctgtttccagtcggtagatattccacaaaacagcagggaagcagcgcttttccgctgcataaccctgcttcggggtcattatagcgattttttcggtatatccatcctttttcgcacgatatacaggattttgccaaagggttcgtgtagactttccttggtgtatccaacggcgtcagccgggcaggataggtgaagtaggcccacccgcgagcgggtgttccttcttcactgtcccttattcgcacctggcggtgctcaacgggaatcctgctctgcgaggctggccggctaccgccggcgtaacagatgagggcaagcggatggctgatgaaaccaagccaaccaggaagggcagcccacctatcaaggtgtactgccttccagacgaacgaagagcgattgaggaaaaggcggcggcggccggcatgagcctgtcggcctacctgctggccgtcggccagggctacaaaatcacgggcgtcgtggactatgagcacgtccgcgagggcgtcccggaaaacgattccgaagcccaacctttcatagaaggcggcggtggaatcgaaatctcgtgatggcaggttgggcgtcgcttggtcggtcatttcgaaaaaggttaggaatacggttagccatttgcctgcttttatatagttcantatgggattcacctttatgttgataagaaataaaagaaaatgccaataggatatcggcattttcttttgcgtttttatttgttaactgttaattgtccttgttcaaggatgctgtctttgacaacagatgttttcttgcctttgatgttcagcaggaagctcggcgcaaacgttgattgtttgtctgcgtagaatcctctgtttgtcatatagcttgtaatcacgacattgtttcctttcgcttgaggtacagcgaagtgtgagtaagtaaaggttacatcgttaggcggatcaagatccatttttaacacaaggccagttttgttcagcggcttgtatgggccagttaaagaattagaaacataaccaagcatgtaaatatcgttagacgtaatgccgtcaatcgtcatttttgatccgcgggagtcagtgaacaggtaccatttgccgttcattttaaagacgttcgcgcgttcaatttcatctgttactgtgttagatgcaatcagcggtttcatcacttttttcagtgtgtaatcatcgtttagctcaatcataccgagagcgccgtttgctaactcagccgtgcgttttttatcgctttgcagaagtttttgactttcttgacggaagaatgatgtgcttttgccatagtatgctttgttaaataaagattcttcgccttggtagccatcttcagttccagtgtttgcttcaaatactaagtatttgtggcctttatcttctacgtagtgaggatctctcagcgtatggttgtcgcctgagctgtagttgccttcatcgatgaactgctgtacattttgatacgtttttccgtcaccgtcaaagattgatttataatcctctacaccgttgatgttcaaagagctgtctgatgctgatacgttaacttgtgcagttgtcagtgtttgtttgccgtaatgtttaccggagaaatcagtgtagaataaacggatttttccgtcagatgtaaatgtggctgaacctgaccattcttgtgtttggtcttttaggatagaatcatttgcatcgaatttgtcgctgtctttaaagacgcggccagcgtttttccagctgtcaatagaagtttcgccgactttttgatagaacatgtaaatcgatgtgtcatccgcatttttaggatctccggctaatgcaaagacgatgtggtagccgtgatagtttgcgacagtgccgtcagcgttttgtaatggccagctgtcccaaacgtccaggccttttgcagaagagatatttttaattgtggacgaatcaaattcagaaacttgatatttttcatttttttgctgttcagggatttgcagcatatcatggcgtgtaatatgggaaatgccgtatgtttccttatatggcttttggttcgtttctttcgcaaacgcttgagttgcgcctcctgccagcagtgcggtagtaaaggttaatactgttgcttgttttgcaaactttttgatgttcatcgttcatgtctccttttttatgtactgtgttagcggtctgcttcttccagccctcctgtttgaagatggcaagttagttacgcacaataaaaaaagacctaaaatatgtaaggggtgacgccaaagtatacactttgccctttacacattttaggtcttgcctgctttatcagtaacaaacccgcgcgatttacttttcgacctcattctattagactctcgtttggattgcaactggtctattttcctcttttgtttgatagaaaatcataaaaggatttgcagactacgggcctaaagaactaaaaaatctatctgtttcttttcattctctgtattttttatagtttctgttgcatgggcataaagttgcctttttaatcacaattcagaaaatatcataatatctcatttcactaaataatagtgaacggcaggtatatgtgatgggttaaaaaggatcaccccagagtcccgctcagaagaactcgtcaagaaggcgatagaaggcgatgcgctgcgaatcgggagcggcgataccgtaaagcacgaggaagcggtcagcccattcgccgccaagctcttcagcaatatcacgggtagccaacgctatgtcctgatagcggtccgccacacccagccggccacagtcgatgaatccagaaaagcggccattttccaccatgatattcggcaagcaggcatcgccatgggtcacgacgagatcctcgccgtcgggcatccgcgccttgagcctggcgaacagttcggctggcgcgagcccctgatgctcttcgtccagatcatcctgatcgacaagaccggcttccatccgagtacgtgctcgctcgatgcgatgtttcgcttggtggtcgaatgggcaggtagccggatcaagcgtatgcagccgccgcattgcatcagccatgatggatactttctcggcaggagcaaggtgagatgacaggagatcctgccccggcacttcgcccaatagcagccagtcccttcccgcttcagtgacaacgtcgagacagctgcgcaaggaacgcccgtcgtggccagccacgatagccgcgctgcctcgtcttggagttcattcagggcaccggacaggtcggtcttgacaaaaagaaccgggcgcccctgcgctgacagccggaacacggcggcatcagagcagccgattgtctgttgtgcccagtcatagccgaatagcctctccacccaagcggccggagaacctgcgtgcaatccatcttgttcaatcatgcgaaacgatcctcatcctgtctcttgatcagatcttgatcccctgcgccatcagatccttggcggcaagaaagccatccagtttactttgcagggcttcccaaccttaccagagggcgccccagctggcaattccg